European Patent Application EP 4 180 516 A1, published May 17, 2023. Title: Skeletal muscle progenitor cells and Method for purifying same, Composition for treating myogenic disease, and Method for producing cell group comprising skeletal muscle progenitor cells. Applicant: ASAHI KASEI KABUSHIKI KAISHA KYOTO UNIVERSITY. Application 2020-120226. The sequence listing filed with the application follows.

SEQUENCE LISTING (10 sequences)

SEQ ID NO: 1 - DNA, 20 bp, Artificial Sequence
  Oligonucleotide
agggcctcctgcttgtttat

SEQ ID NO: 2 - DNA, 20 bp, Artificial Sequence
  Oligonucleotide
ggttttgcccaactcagtgt

SEQ ID NO: 3 - DNA, 20 bp, Artificial Sequence
  Oligonucleotide
cactccggtcccaaatgtag

SEQ ID NO: 4 - DNA, 20 bp, Artificial Sequence
  Oligonucleotide
ttccctgtagcaccacacac

SEQ ID NO: 5 - DNA, 20 bp, Artificial Sequence
  Oligonucleotide
agggcctcggtgagatagtt

SEQ ID NO: 6 - DNA, 20 bp, Artificial Sequence
  Oligonucleotide
aagagttcaccgacctgctg

SEQ ID NO: 7 - DNA, 20 bp, Artificial Sequence
  Oligonucleotide
ggccccatttacatcatcac

SEQ ID NO: 8 - DNA, 20 bp, Artificial Sequence
  Oligonucleotide
catagctccgtgtgctttca

SEQ ID NO: 9 - DNA, 19 bp, Artificial Sequence
  Oligonucleotide
ctcttccagccttccttcc

SEQ ID NO: 10 - DNA, 20 bp, Artificial Sequence
  Oligonucleotide
caccttcaccgttccagttt